European Patent Specification EP 4 018 004 B1, published June 18, 2025. Title: COMPOSITIONS, METHODS AND KITS FOR DETECTING TREPONEMA PALLIDUM. Applicant: GEN-PROBE INCORPORATED O'DONNELL, Meghan A. DARBY, Paul M. GETMAN, Damon K. The sequence listing filed with the application follows.

SEQUENCE LISTING (39 sequences)

SEQ ID NO: 1 - RNA, 114 nt, Treponema pallidum
gcacauguccugugauccggggaugaccgaaugggguaacccgacaggguaaagccuugucauugccuuccugaaugaauagggaggguaaggcgaaacugggugaacugaacc

SEQ ID NO: 2 - RNA, 131 nt, Treponema denticola
uccugugauacggaaauagccgaaugggguaacccguuaguagugauacugacauuacgcucuugaauaaaauagagagguaaagcgauacugagugaacugaaccaucuaaguaacucaaggaaaagaaa

SEQ ID NO: 3 - DNA, 31 bp, Treponema pallidum
ggttcagttcacccagtttcgccttaccctc

SEQ ID NO: 4 - DNA, 27 bp, Treponema pallidum
cagttcacccagtttcgccttaccctc

SEQ ID NO: 5 - DNA, 22 bp, Treponema pallidum
ggttcagttcacccagtttcgc

SEQ ID NO: 6 - DNA, 19 bp, Treponema pallidum
ccagtttcgccttaccctc

SEQ ID NO: 7 - DNA, 18 bp, Treponema pallidum
cagttcacccagtttcgc

SEQ ID NO: 8 - DNA, 22 bp, Treponema pallidum
ggttcagttcacccagtttcgc

SEQ ID NO: 9 - DNA, 27 bp, Artificial Sequence
  T7 phage promoter
aatttaatacgactcactatagggaga

SEQ ID NO: 10 - DNA, 46 bp, Artificial Sequence
  T7 promoter primer
aatttaatacgactcactatagggagaccagtttcgccttaccctc

SEQ ID NO: 11 - DNA, 45 bp, Artificial Sequence
  T7 promoter primer
aatttaatacgactcactatagggagacagttcacccagtttcgc

SEQ ID NO: 12 - DNA, 49 bp, Artificial Sequence
  T7 promoter primer
aatttaatacgactcactatagggagaggttcagttcacccagtttcgc

SEQ ID NO: 13 - DNA, 61 bp, Treponema pallidum
gcacatgtcctgtgatccggggatgaccgaatggggtaacccgacagggtaaagccttgtc

SEQ ID NO: 14 - DNA, 52 bp, Treponema pallidum
ctgtgatccggggatgaccgaatggggtaacccgacagggtaaagccttgtc

SEQ ID NO: 15 - DNA, 29 bp, Treponema pallidum
gcacatgtcctgtgatccggggatgaccg

SEQ ID NO: 16 - DNA, 20 bp, Treponema pallidum
cgacagggtaaagccttgtc

SEQ ID NO: 17 - DNA, 20 bp, Treponema pallidum
ctgtgatccggggatgaccg

SEQ ID NO: 18 - DNA, 17 bp, Treponema pallidum
gcacatgtcctgtgatc

SEQ ID NO: 19 - DNA, 47 bp, Treponema pallidum
cccgacagggtaaagccttgtcattgccttcctgaatgaatagggag

SEQ ID NO: 20 - DNA, 27 bp, Treponema pallidum
cccgacagggtaaagccttgtcattgc

SEQ ID NO: 21 - DNA, 33 bp, Treponema pallidum
gccttgtcattgccttcctgaatgaatagggag

SEQ ID NO: 22 - RNA, 13 nt, Treponema pallidum
  misc_feature (1)..(13): Backbone includes 2'-O-methyl analogs
gccuuccugaaug

SEQ ID NO: 23 - RNA, 14 nt, Treponema pallidum
  misc_feature (1)..(14): Backbone includes 2'-O-methyl analogs
cgacaggguaaagc

SEQ ID NO: 24 - RNA, 16 nt, Treponema pallidum
  misc_feature (1)..(16): Backbone includes 2'-O-methyl analogs
ccgacaggguaaagcc

SEQ ID NO: 25 - RNA, 16 nt, Treponema pallidum
  misc_feature (1)..(16): Backbone includes 2'-O-methyl analogs
cccgacaggguaaagc

SEQ ID NO: 26 - RNA, 13 nt, Treponema pallidum
  misc_feature (1)..(13): Backbone includes 2'-O-methyl analogs
gccuugucauugc

SEQ ID NO: 27 - RNA, 22 nt, Treponema pallidum
  misc_feature (1)..(22): Backbone includes 2'-O-methyl analogs
gccuuccugaaugaauagggag

SEQ ID NO: 28 - RNA, 17 nt, Artificial Sequence
  Molecular torch hybridization probe
  misc_feature (1)..(17): Backbone includes 2'-O-methyl analogs
  misc_feature (1)..(17): 5' fluorophore/3' quencher
  misc_feature (13)..(14): C9 linker between bases 13/14
gccuuccugaaugaggc

SEQ ID NO: 29 - RNA, 18 nt, Artificial Sequence
  Molecular torch hybridization probe
  misc_feature (1)..(18): Backbone includes 2'-O-methyl analogs
  misc_feature (1)..(18): 5' fluorophore/3' quencher
  misc_feature (14)..(15): C9 linker between bases 14/15
cgacaggguaaagcgucg

SEQ ID NO: 30 - RNA, 21 nt, Artificial Sequence
  Molecular torch hybridization probe
  misc_feature (1)..(21): Backbone includes 2'-O-methyl analogs
  misc_feature (1)..(21): 5' fluorophore/3' quencher
  misc_feature (16)..(17): C9 linker between bases 16/17
ccgacaggguaaagccgucgg

SEQ ID NO: 31 - RNA, 21 nt, Artificial Sequence
  Molecular torch hybridization probe
  misc_feature (1)..(21): Backbone includes 2'-O-methyl analogs
  misc_feature (1)..(21): 5' fluorophore/3' quencher
  misc_feature (16)..(17): C9 linker between bases 16/17
cccgacaggguaaagcucggg

SEQ ID NO: 32 - RNA, 17 nt, Artificial Sequence
  Molecular torch hybridization probe
  misc_feature (1)..(17): Backbone includes 2'-O-methyl analogs
  misc_feature (1)..(17): 5' fluorophore/3' quencher
  misc_feature (13)..(14): C9 linker between bases 13/14
gccuugucauugcaggc

SEQ ID NO: 33 - RNA, 26 nt, Artificial Sequence
  Molecular torch hybridization probe
  misc_feature (1)..(26): Backbone includes 2'-O-methyl analogs
  misc_feature (1)..(26): 5' fluorophore/3' quencher
  misc_feature (22)..(23): C9 linker between bases 22/23
gccuuccugaaugaauagggagaggc

SEQ ID NO: 34 - RNA, 27 nt, Treponema pallidum
  misc_feature (1)..(27): Backbone includes 2'-O-methyl analogs
gcaagcccgcgcggcccuacaaccccu

SEQ ID NO: 35 - RNA, 19 nt, Treponema pallidum
  misc_feature (1)..(19): Backbone includes 2'-O-methyl analogs
cgguacuuguccacuaucg

SEQ ID NO: 36 - RNA, 22 nt, Treponema pallidum
  misc_feature (1)..(22): Backbone includes 2'-O-methyl analogs
cgguaguugucgaguauuuagc

SEQ ID NO: 37 - DNA, 60 bp, Artificial Sequence
  Target capture oligonucleotide
  misc_feature (1)..(27): Target-complementary sequence
  misc_feature (1)..(27): Backbone includes 2'-O-methyl analogs
gcaagcccgcgcggcccuacaaccccutttaaaaaaaaaaaaaaaaaaaaaaaaaaaaaa

SEQ ID NO: 38 - DNA, 52 bp, Artificial Sequence
  Target capture oligonucleotide
  misc_feature (1)..(19): Target-complementary sequence
  misc_feature (1)..(19): Backbone includes 2'-O-methyl analogs
cgguacuuguccacuaucgtttaaaaaaaaaaaaaaaaaaaaaaaaaaaaaa

SEQ ID NO: 39 - DNA, 55 bp, Artificial Sequence
  Target capture oligonucleotide
  misc_feature (1)..(22): Target-complementary sequence
  misc_feature (1)..(22): Backbone includes 2'-O-methyl analogs
cgguaguugucgaguauuuagctttaaaaaaaaaaaaaaaaaaaaaaaaaaaaaa